European Patent Application EP 4 174 083 A1, published May 3, 2023. Title: NEUTRALIZING MONOCLONAL ANTIBODIES AGAINST SARBECOVIRUSES. Applicant: Ospedale San Raffaele s.r.l. The sequence listing filed with the application follows.

SEQUENCE LISTING (88 sequences)

SEQ ID NO: 1 - protein, 8 aa, Artificial sequence
  CDR1 sequence of the heavy chain variable region
GFNFNTYT

SEQ ID NO: 2 - protein, 10 aa, Artificial sequence
  CDR1 sequence of the heavy chain variable region
GGSISSINYY

SEQ ID NO: 3 - protein, 10 aa, Artificial sequence
  CDR1 sequence of the heavy chain variable region
GDSVSRRSVA

SEQ ID NO: 4 - protein, 10 aa, Artificial sequence
  CDR1 sequence of the heavy chain variable region
GGSISSRNFY

SEQ ID NO: 5 - protein, 8 aa, Artificial sequence
  CDR2 sequence of the heavy chain variable region
ISSSSSYI

SEQ ID NO: 6 - protein, 7 aa, Artificial sequence
  CDR2 sequence of the heavy chain variable region
INYSGTT

SEQ ID NO: 7 - protein, 9 aa, Artificial sequence
  CDR2 sequence of the heavy chain variable region
TYYRSKWFS

SEQ ID NO: 8 - protein, 7 aa, Artificial sequence
  CDR2 sequence of the heavy chain variable region
IYTSGST

SEQ ID NO: 9 - protein, 25 aa, Artificial sequence
  CDR3 sequence of the heavy chain variable region
TRVNPQAKGSDWLDPPINQYYGMDV

SEQ ID NO: 10 - protein, 20 aa, Artificial sequence
  CDR3 sequence of the heavy chain variable region
ARQTYYYDRRGYYRPEPIEH

SEQ ID NO: 11 - protein, 18 aa, Artificial sequence
  CDR3 sequence of the heavy chain variable region
RKSKGRQQLAESTSSVWT

SEQ ID NO: 12 - protein, 20 aa, Artificial sequence
  CDR3 sequence of the heavy chain variable region
ARGTFYYDRSGNGRLDPLDY

SEQ ID NO: 13 - protein, 7 aa, Artificial sequence
  CDR1 sequence of the light chain variable region
QSVSSSY

SEQ ID NO: 14 - protein, 6 aa, Artificial sequence
  CDR1 sequence of the light chain variable region
QDVRSF

SEQ ID NO: 15 - protein, 6 aa, Artificial sequence
  CDR1 sequence of the light chain variable region
QGIRND

SEQ ID NO: 16 - protein, 6 aa, Artificial sequence
  CDR1 sequence of the light chain variable region
QDISNY

SEQ ID NO: 17 - DNA, 22 bp, Artificial sequence
  Forward primer for the amplification of the heavy chain VH135
aggtgcagctgctcgagtctgg

SEQ ID NO: 18 - DNA, 29 bp, Artificial sequence
  Reverse primer or the amplification of heavy chain of IgG1
gcatgtactagttttgtcacaagatttgg

SEQ ID NO: 19 - DNA, 23 bp, Artificial sequence
  Forward primer for the amplification of VH2
cagatcaccttgctcgagtctgg

SEQ ID NO: 20 - protein, 9 aa, Artificial sequence
  CDR3 sequence of the light chain variable region
QQYGSSPWT

SEQ ID NO: 21 - protein, 5 aa, Artificial sequence
  CDR3 sequence of the light chain variable region
QQYVT

SEQ ID NO: 22 - protein, 9 aa, Artificial sequence
  CDR3 sequence of the light chain variable region
QQTYDTPLT

SEQ ID NO: 23 - protein, 9 aa, Artificial sequence
  CDR3 sequence of the light chain variable region
LQDYNFPRT

SEQ ID NO: 24 - protein, 8 aa, Artificial sequence
  CDR3 sequence of the light chain variable region
QQHDNLVT

SEQ ID NO: 25 - protein, 21 aa, Artificial sequence
  FR1 sequence of the heavy chain variable region
LESGGGLVKPGGSLRLSCAAS

SEQ ID NO: 26 - protein, 21 aa, Artificial seqeunce
  FR1 sequence of the heavy chain variable region
LEWGPGLVKPSETLSLTCTVS

SEQ ID NO: 27 - protein, 21 aa, Artificial sequence
  FR1 sequence of the heavy chain variable sequence
LESGPGLLKPSQSLSLTCAIS

SEQ ID NO: 28 - protein, 21 aa, Artificial sequence
  FR1 sequence of the heavy chain variable region
LEWGPGLVKASQTLSLTCTVS

SEQ ID NO: 29 - protein, 17 aa, Artificial sequence
  FR2 sequence of the heavy chain variable region
MNWVRQAPGKGLEWVSS

SEQ ID NO: 30 - protein, 17 aa, Artificial sequence
  FR2 sequence of the heavy chain variable region
WVWIRQPPGKGLEWIGN

SEQ ID NO: 31 - protein, 17 aa, Artificial sequence
  FR2 sequence of the heavy chain variable region
WNWIRQSPSRGLEWLGR

SEQ ID NO: 32 - protein, 17 aa, Artificial sequence
  FR2 sequence of the heavy chain variable region
WSWIRQPGGKGLEWIGR

SEQ ID NO: 33 - protein, 38 aa, Artificial sequence
  FR3 sequence of the heavy chain variable region
DNADSVKGRFTIYRDNAKKSLYLRMIGLRVEDSGVYYC

SEQ ID NO: 34 - protein, 38 aa, Artificial sequence
  FR3 sequence of the heavy chain variable region
NYNPSLKSRVTISVDTSKNQFSLKLSSVTAADTAVYYC

SEQ ID NO: 35 - protein, 38 aa, Artificial sequence
  FR3 sequence of the heavy chain variable region
EYGVSVRGRITISPDTTKNQFSLQLNSVTPEDTAVYYC

SEQ ID NO: 36 - protein, 38 aa, Artificial sequence
  FR3 sequence of the heavy chain variable region
NYNPSLKSRVTISLDTSKSQFSLKLSSVTAADTAVYYC

SEQ ID NO: 37 - protein, 11 aa, Artificial sequence
  FR4 sequence of the heavy chain variable region
WGQGTTVTVSS

SEQ ID NO: 38 - protein, 11 aa, Artificial sequence
  FR4 sequence of the heavy chain variable region
WGQRDHGHRSP

SEQ ID NO: 39 - protein, 11 aa, Artificial sequence
  FR4 sequence of the heavy chain variable region
WGQGTLVTVSS

SEQ ID NO: 40 - protein, 11 aa, Artificial sequence
  FR4 sequence of the heavy chain variable region
WGQGTTVIVYS

SEQ ID NO: 41 - protein, 26 aa, Artificial sequence
  FR1 sequence of the light chain variable region
ELTLTQSPGTLSLSPGERATLSCRAS

SEQ ID NO: 42 - protein, 26 aa, Artificial sequence
  FR1 sequence of the light chain variable region
ELTLTQSPATLSLSPGDRATLSCRAS

SEQ ID NO: 43 - protein, 26 aa, Artificial sequence
  FR1 sequence of the light chain variable region
ELVMTQSPSFLSASVGDRVTITCRAS

SEQ ID NO: 44 - protein, 26 aa, Artificial sequence
  FR1 sequence of the light chain variable region
ELVMTQSPSSLSAFVGDRVTLTCRAS

SEQ ID NO: 45 - protein, 26 aa, Artificial sequence
  FR1 sequence of the light chain variable region
ELVMTQSPSSLSASVGDRVTITCQAS

SEQ ID NO: 46 - protein, 17 aa, Artificial sequence
  FR2 sequence of the light chain variable region
LAWYQQKPGQAPRLLIY

SEQ ID NO: 47 - protein, 17 aa, Artificial sequence
  FR2 sequence of the light chain variable region
LAWYQHKPGQPPRLLIY

SEQ ID NO: 48 - protein, 17 aa, Artificial sequence
  FR2 sequence of the light chain variable region
LHWYQQRPGKAPKLLIY

SEQ ID NO: 49 - protein, 17 aa, Artificial sequence
  FR2 sequence of the light chain variable region
LNWYQQKPGQPPKLLIY

SEQ ID NO: 50 - protein, 17 aa, Artificial sequence
  FR2 sequence of the light chain variable region
LNWYQQKPGKAPKLLIY

SEQ ID NO: 51 - protein, 36 aa, Artificial sequence [sequence omitted]

SEQ ID NO: 52 - protein, 36 aa, Artificial sequence
  FR3 sequence of the light chain variable region
SRAAGIPDRFSGSGSGTDFTLTISRLEPEDFAVYYC

SEQ ID NO: 53 - protein, 36 aa, Artificial sequence
  FR3 sequence of the light chain variable region
MVSSEVPSRFSGSGSETDFTLTIDGLQPEDVATYFC

SEQ ID NO: 54 - protein, 36 aa, Artificial sequence
  FR3 sequence of the light chain variable region
ALQSGVPSRFSGSGFGTDFTLTISSLQPEDIATYYC

SEQ ID NO: 55 - protein, 36 aa, Artificial sequence
  FR3 sequence of the light chain variable region
NLETGVPSRFSGSGFGTHFTLTISSLQPEDFATYYC

SEQ ID NO: 56 - protein, 10 aa, Artificial sequence
  FR4 sequence of the light chain variable region
FGQGTKVEIK

SEQ ID NO: 57 - protein, 10 aa, Artificial sequence
  FR4 sequence of the light chain variable region
FGPGTKVDIK

SEQ ID NO: 58 - protein, 10 aa, Artificial sequence
  FR4 sequence of the light chain variable region
FGGGTAVDIK

SEQ ID NO: 59 - protein, 10 aa, Artificial sequence
  FR4 sequence of the light chain variable region
FGGGTKVEIK

SEQ ID NO: 60 - protein, 128 aa, Artificial sequence
  Fab#5 heavy chain variable sequence
LESGGGLVKPGGSLRLSCAASGFNFNTYTMNWVRQAPGKGLEWVSSISSSSSYIDNADSVKGRFTIYRDNAKKSLYLRMIGLRVEDSGVYYCTRVNPQAKGSDWLDPPINQYYGMDVWGQGTTVTVSS

SEQ ID NO: 61 - protein, 108 aa, Artificial sequence
  Fab#5 light chain variable sequence
ELTLTQSPGTLSLSPGERATLSCRASQSVSSSYLAWYQQKPGQAPRLLIYGASSRATGIPDRFSGSGSGTDFTLTISRLEPEDFAVYYCQQYGSSPWTFGQGTKVEIK

SEQ ID NO: 62 - protein, 128 aa, Artificial sequence
  BU2 heavy chain variable sequence
LESGGGLVKPGGSLRLSCAASGFNFNTYTMNWVRQAPGKGLEWVSSISSSSSYIDNADSVKGRFTIYRDNAKKSLYLRMIGLRVEDSGVYYCTRVNPQAKGSDWLDPPINQYYGMDVWGQRDHGHRSP

SEQ ID NO: 63 - protein, 104 aa, Artificial sequence
  BU2 light chain variable sequence
ELTLTQSPATLSLSPGDRATLSCRASQSVSSSYLAWYQHKPGQPPRLLIYGASSRAAGIPDRFSGSGSGTDFTLTISRLEPEDFAVYYCQQYVTFGPGTKVDIK

SEQ ID NO: 64 - protein, 124 aa, Artificial sequence
  BU7 heavy chain variable sequence
LEWGPGLVKPSETLSLTCTVSGGSISSINYYWVWIRQPPGKGLEWIGNINYSGTTNYNPSLKSRVTISVDTSKNQFSLKLSSVTAADTAVYYCARQTYYYDRRGYYRPEPIEHWGQGTLVTVSS

SEQ ID NO: 65 - protein, 107 aa, Artificial sequence
  BU7 light chain variable sequence
ELVMTQSPSFLSASVGDRVTITCRASQDVRSFLHWYQQRPGKAPKLLIYAASMVSSEVPSRFSGSGSETDFTLTIDGLQPEDVATYFCQQTYDTPLTFGGGTAVDIK

SEQ ID NO: 66 - protein, 124 aa, Artificial sequence
  BU11 heavy chain variable sequence
LESGPGLLKPSQSLSLTCAISGDSVSRRSVAWNWIRQSPSRGLEWLGRTYYRSKWFSEYGVSVRGRITISPDTTKNQFSLQLNSVTPEDTAVYYCRKSKGRQQLAESTSSVWTWGQGTTVIVYS

SEQ ID NO: 67 - protein, 107 aa, Artificial sequence
  BU11 light chain variable sequence
ELVMTQSPSSLSAFVGDRVTLTCRASQGIRNDLNWYQQKPGQPPKLLIYAASALQSGVPSRFSGSGFGTDFTLTISSLQPEDIATYYCLQDYNFPRTFGQGTKVEIK

SEQ ID NO: 68 - protein, 123 aa, Artificial sequence
  BU54 heavy chain variable sequence
LEWGPGLVKASQTLSLTCTVSGGSISSRNFYWSWIRQPGGKGLEWIGRIYTSGSTNYNPSLKSRVTISLDTSKSQFSLKLSSVTAADTAVYYCARGTFYYDRSGNGRLDPLDYWGQGTLVTVS

SEQ ID NO: 69 - protein, 106 aa, Artificial sequence
  BU54 light chain variable sequence
ELVMTQSPSSLSASVGDRVTITCQASQDISNYLNWYQQKPGKAPKLLIYDASNLETGVPSRFSGSGFGTHFTLTISSLQPEDFATYYCQQHDNLVTFGGGTKVEIK

SEQ ID NO: 70 - DNA, 384 bp, Artificial sequence
  DNA sequence encoding for the heavy chain variable region of clone Fab#5
ctcgagtctgggggaggcctggtcaagcctggggggtccctgagactctcctgtgcagcctctggattcaacttcaatacctataccatgaactgggtccgccaggctccagggaaggggctggagtgggtctcatccattagtagtagtagtagttacatagacaacgcagactcagtgaagggccgattcaccatctacagagacaacgccaagaagtcactgtatctgcgaatgatcggcctgagagtcgaggactccggtgtgtattactgtacgcgagtgaacccccaggccaaagggtcggactggttggatccccccatcaaccaatactacggtatggacgtctggggccaagggaccacggtcaccgtctcctca

SEQ ID NO: 71 - DNA, 324 bp, Artificial sequence
  DNA sequence encoding for the light chain variable region of clone Fab#5
gagctcacactcacgcagtctccaggcaccctgtctttgtctccaggggaaagagccaccctctcctgcagggccagtcagagtgttagcagcagctatttagcctggtaccagcagaaacctggccaggctcccaggctcctcatctatggtgcatccagcagggccactggcatcccagacaggttcagtggcagtgggtctgggacagacttcactctcaccatcagcagactggagcctgaagattttgcagtgtattactgtcagcagtatggtagctcaccgtggacgttcggccaagggaccaaggttgaaatcaaa

SEQ ID NO: 72 - DNA, 384 bp, Artificial sequence
  DNA sequence encoding for the heavy chain variable region of clone Fab BU.2
ctcgagtctgggggaggcctggtcaagcctggggggtccctgagactctcctgtgcagcctctggattcaacttcaatacctataccatgaactgggtccgccaggctccagggaaggggctggagtgggtctcatccattagtagtagtagtagttacatagacaacgcagactcagtgaagggccgattcaccatctacagagacaacgccaagaagtcactgtatctgcgaatgatcggcctgagagtcgaggactccggtgtgtattactgtacgcgagtgaacccccaggccaaagggtcggactggttggatccccccatcaaccaatactacggtatggacgtctggggccaaagggaccacggtcaccggtctcct

SEQ ID NO: 73 - DNA, 312 bp, Artificial sequence
  DNA sequence encoding for the light chain variable region of clone Fab BU.2
gagctcacactcacgcagtctccagccaccctgtctttgtctccaggggatagagccaccctctcctgcagggccagtcagagtgttagcagcagttacttagcctggtaccagcacaaacctggccagccccccaggctcctcatctatggtgcatccagcagggccgccggcatcccagacaggttcagtggcagtgggtctgggacagacttcactctcaccatcagcagactggagcctgaagattttgcagtgtattactgtcagcagtacgtcactttcggccctgggaccaaagtggatatcaaa

SEQ ID NO: 74 - DNA, 372 bp, Artificial sequence
  DNA sequence encoding for the heavy chain variable region of clone Fab BU.7
ctcgagtggggcccaggactggtgaagccttcggagaccctgtccctcacctgcactgtctctggtggctccatcagcagcataaattactactgggtctggattcgccagcccccagggaaggggctggagtggattgggaatatcaattacagtgggaccaccaactacaacccgtccctcaagagtcgagtcaccatatccgtggacacgtccaagaaccagttctccctgaagctgagctctgtgaccgccgcagacacggctgtctattactgtgcgagacaaacgtattactatgataggcgtggttattaccgcccggagcccattgagcactggggccagggaaccctggtcaccgtctcctca

SEQ ID NO: 75 - DNA, 321 bp, Artificial sequence
  DNA sequence encoding for the light chain variable region of clone Fab BU.7
gagctcgtgatgacacagtctccatccttcctgtctgcatctgtaggagacagagtcaccatcacttgccgggcaagtcaagatgttagaagttttttacattggtatcaacaaagaccagggaaagcccctaagttgttgatctatgctgcatccatggtgtcgagtgaggtcccgtcaaggttcagtggcagtggatctgagacagatttcactctcaccatcgacggtctgcaacctgaagatgttgcaacttacttctgtcaacagacttacgacacgccgctcaccttcggcggcgggaccgcggttgacatcaaa

SEQ ID NO: 76 - DNA, 372 bp, Artificial sequence
  DNA sequence encoding for the heavy chain variable region of clone Fab BU.11
ctcgagtcaggtccaggactgctgaagccctcgcagagcctctcactcacctgtgccatctccggagacagtgtctctaggagaagtgttgcttggaactggatcagacagtccccatcgagaggccttgagtggctgggaaggacatactacaggtccaagtggttttctgagtatggcgtatctgtgagaggtcgaataaccatcagtccagacacaaccaagaaccagttctccctgcagctgaactccgtgactcccgaggacacggctgtctattactgtcgaaagtcgaaagggaggcagcagttggcagagtctacgagttcggtatggacgtggggccaagggaccacggtcatcgtctactca

SEQ ID NO: 77 - DNA, 321 bp, Artificial sequence
  DNA sequence encoding for the light chain variable region of clone Fab BU.11
gagctcgtgatgacacagtctccatcctccctgtctgcatttgtgggagatagagtcaccctcacttgccgggcaagtcagggcattagaaatgatttaaactggtatcagcagaaaccagggcaaccccctaaactcctgatctatgctgcatccgctttacaaagtggcgtcccatcaaggttcagcggcagtgggtttggcacagatttcactctcaccatcagcagcctgcagcctgaagatattgcaacttattactgtctacaagattacaatttccctcggacgttcggccaagggaccaaggtggaaatcaaa

SEQ ID NO: 78 - DNA, 372 bp, Artificial sequence
  DNA sequence encoding for the heavy chain variable region of clone Fab BU.54
ctcgagtggggcccaggactggtgaaggcttcacagaccctgtccctcacctgcactgtctctggtggctccatcagcagtaggaatttctattggagttggatccggcagcccggcgggaagggactggagtggattgggcgtatctatacaagtgggagcaccaattacaatccctccctcaagagtcgagtcactatatcattagacacgtccaagagtcagttctccctgaagctgagctctgtgaccgccgcagacacggccgtgtattattgtgcgagagggacgttttattatgataggagtggtaatggtcgattagatccgcttgactactggggccagggaaccctggtcaccgtctcctca

SEQ ID NO: 79 - DNA, 318 bp, Artificial sequence
  DNA sequence encoding for the light chain variable region of clone Fab BU.54
gagctcgtgatgacacagtctccatcctccctgtctgcatctgtaggagacagagtcaccatcacttgccaggcgagtcaggacattagcaactatttaaattggtatcagcagaaaccagggaaagcccctaagctcctgatctacgatgcatccaatttggaaacaggggtcccatcaaggttcagtggaagtggatttgggacacattttacgttaaccatcagcagcctgcagcctgaagattttgcaacatattactgtcaacagcatgataatctcgtcactttcggcggagggaccaaggtggagatcaaa

SEQ ID NO: 80 - DNA, 23 bp, Artificial sequence
  Forward primer for amplification of the heavy chain
caggtgcagctgctcgagtcggg

SEQ ID NO: 81 - DNA, 23 bp, Artificial sequence
  Forward primer for amplification of the heavy chain
caggtgcagctactcgagtgggg

SEQ ID NO: 82 - DNA, 24 bp, Artificial sequence
  Forward primer for the amplification of the heavy chain
caggtgcagctactcgagtggggc

SEQ ID NO: 83 - DNA, 23 bp, Artificial sequence
  Forward primer for the amplification of the heavy chain
caggtacagctgctcgagtcagg

SEQ ID NO: 84 - DNA, 38 bp, Artificial sequence
  Forward primer for the amplification of the light chain
gagccgcacgagcccgagctccagatgacccagtctcc

SEQ ID NO: 85 - DNA, 58 bp, Artificial sequence
  Reverse primer for the amplification of the light chain
gcgccgtctagaattaacactctcccctgttgaagctctttgtgacgggcgaactcag

SEQ ID NO: 86 - DNA, 38 bp, Artificial sequence
  Forward primer for the amplification of the light chain
gagccgcacgagcccgagctcgtgatgacacagtctcc

SEQ ID NO: 87 - DNA, 38 bp, Artificial sequence
  Forward primer for the amplification of the heavy chain
gagccgcacgagcccgagctcgtgatgacccagtctcc

SEQ ID NO: 88 - DNA, 38 bp, Artificial sequence
  Forward primer for the amplification of the light chain
gagccgcacgagcccgagctcacactcacgcagtctcc